European Patent Specification EP 3 995 588 B1, published December 17, 2025. Title: LIBRARY PREPARATION METHOD AND APPLICATION. Applicant: GENETRON HEALTH (BEIJING) CO, LTD. The sequence listing filed with the application follows.

SEQUENCE LISTING (33 sequences)

SEQ ID NO: 1 - DNA, 17 bp, Artificial sequence
ggcacccgagaattcca

SEQ ID NO: 2 - DNA, 30 bp, Artificial sequence
ccatctcatccctgcgtgtctccgactcag

SEQ ID NO: 3 - DNA, 10 bp, Artificial sequence
tcctcgaatc

SEQ ID NO: 4 - DNA, 10 bp, Artificial sequence
taggtggttc

SEQ ID NO: 5 - DNA, 10 bp, Artificial sequence
tctaacggac

SEQ ID NO: 6 - DNA, 10 bp, Artificial sequence
ttggagtgtc

SEQ ID NO: 7 - DNA, 10 bp, Artificial sequence
tctagaggtc

SEQ ID NO: 8 - DNA, 10 bp, Artificial sequence
tctggatgac

SEQ ID NO: 9 - DNA, 10 bp, Artificial sequence
tctattcgtc

SEQ ID NO: 10 - DNA, 10 bp, Artificial sequence
aggcaattgc

SEQ ID NO: 11 - DNA, 10 bp, Artificial sequence
ttagtcggac

SEQ ID NO: 12 - DNA, 10 bp, Artificial sequence
cagatccatc

SEQ ID NO: 13 - DNA, 15 bp, Artificial sequence
  misc_feature (1)..(5): n is a, c, g, or t
  misc_feature (9)..(12): n is a, c, g, or t
nnnnnactnnnntga

SEQ ID NO: 14 - DNA, 23 bp, Artificial sequence
caggaacgtactggtgaaaacac

SEQ ID NO: 15 - DNA, 25 bp, Artificial sequence
cttccttctctctctgtcataggga

SEQ ID NO: 16 - DNA, 21 bp, Artificial sequence
ctcccataccctctcagcgta

SEQ ID NO: 17 - DNA, 23 bp, Artificial sequence
cctctctatgggcagtcggtgat

SEQ ID NO: 18 - DNA, 23 bp, Artificial sequence
gaaaatgctggctgacctaaagc

SEQ ID NO: 19 - DNA, 23 bp, Artificial sequence
agcaaagcagaaactcacatcga

SEQ ID NO: 20 - DNA, 21 bp, Artificial sequence
agccatagggcataagctgtg

SEQ ID NO: 21 - DNA, 16 bp, Artificial sequence
ggaggaccgtcgcttg

SEQ ID NO: 22 - DNA, 23 bp, Artificial sequence
gtgagaaagttaaaattcccgtc

SEQ ID NO: 23 - DNA, 18 bp, Artificial sequence
cccataccctctcagcgt

SEQ ID NO: 24 - DNA, 26 bp, Artificial sequence
cttctgcatggtattctttctcttcc

SEQ ID NO: 25 - DNA, 19 bp, Artificial sequence
cacacagcaaagcagaaac

SEQ ID NO: 26 - DNA, 21 bp, Artificial sequence
ccagaaggcgggagacatatg

SEQ ID NO: 27 - DNA, 25 bp, Artificial sequence
actgcagacaagcataaagatgtca

SEQ ID NO: 28 - DNA, 22 bp, Artificial sequence
actactgtagagcccacacctg

SEQ ID NO: 29 - DNA, 20 bp, Artificial sequence
ctgagaacaggctgcagacc

SEQ ID NO: 30 - DNA, 20 bp, Artificial sequence
cctggtgctccatgaggaga

SEQ ID NO: 31 - DNA, 21 bp, Artificial sequence
ctcagcttgtactcagggctc

SEQ ID NO: 32 - DNA, 19 bp, Artificial sequence
actcacgctgcttcccatt

SEQ ID NO: 33 - DNA, 24 bp, Artificial sequence
gtgatccagactctgaccttttgc